European Patent Application EP 4 574 972 A1, published June 25, 2025. Title: Method of specifically increasing lactotransferrin gene expression level and application thereof. Applicant: Qingdao KingAgroot Chemical Compound Co., Ltd. The sequence listing filed with the application follows.

SEQUENCE LISTING (1 sequence)

SEQ ID NO: 1 - protein, 1263 aa, synthetic construct
MNNGTNNFQNFIGISSLQKTLRNALIPTETTQQFIVKNGIIKEDELRGENRQILKDIMDDYYRGFISETLSSIDDIDWTSLFEKMEIQLKNGDNKDTLIKEQTEYRKAIHKKFANDDRFKNMFSAKLISDILPEFVIHNNNYSASEKEEKTQVIKLFSRFATSFKDYFRNRANCFSADDISSSSCHRIVNDNAEIFFSNALVYRRIVKSLSNDDINKISGDMKDSLKEMSLEEIYSYEKYGEFITQEGISFYNDICGKVNSFMNLYCQKNKENKNLYKLQKLHKQILCIADTSYEVPYKFESDEEVYQSVNGFLDNISSKHIVERLRKIGDNYNGYNLDKIYIVSKFYESVSQKTYRDWETINTALEIHYNNILPGNGKSKADKVKKAVKNDLQKSITEINELVSNYKLCSDDNIKAETYIHEISHILNNFEAQELKYNPEIHLVESELKASELKNVLDVIMNAFHWCSVFMTEELVDKDNNFYAELEEIYDEIYPVISLYNLVRNYVTQKPYSTKKIKLNFGIPTLADGWSKSKEYSNNAIILMRDNLYYLGIFNAKNKPDKKIIEGNTSENKGDYKKMIYNLLPGPHKMIPKVFLSSKTGVETYKPSAYILEGYKQNKHIKSSKDFDITFCHDLIDYFKNCIAIHPEWKNFGFDFSDTSTYEDISGFYREVELQGYKIDWTYISEKDIDLLQEKGQLYLFQIYNKDFSKKSTGNDNLHTMYLKNLFSEENLKDIVLKLNGEAEIFFRKSSIKNPIIHKKGSILVNRTYEAEEKDQFGNIQIVRKNIPENIYQELYKYFNDKSDKELSDEAAKLKNVVGHHEAATNIVKDYRYTYDKYFLHMPITINFKANKTGFINDRILQYIAKEKDLHVIGIDRGERNLIYVSVIDTCGNIVEQKSFNIVNGYDYQIKLKQQEGARQIARKEWKEIGKIKEIKEGYLSLVIHEISKMVIKYNAIIAMEDLSYGFKKGRFKVERQVYQKFETMLINKLNYLVFKDISITENGGLLKGYQLTYIPDKLKNVGHQCGCIFYVPAAYTSKIDPTTGFVNIFKFKDLTVDAKREFIKKFDSIRYDSEKNLFCFTFDYNNFITQNTVMSKSSWSVYTYGVRIKRRFVNGRFSNESDTIDITKDMEKTLEMTDINWRDGHDLRQDIIDYEIVQHIFEIFRLTVQMRNSLSELEDRDYDRLISPVLNENNIFYDSAKAGDALPKDADANGAYCIALKGLYEIKQITENWKEDGKFSRDKLKISNKDWFDFIQNKRYL